European Patent Application EP 4 001 305 A9, published May 24, 2023. Title: ANTI-TAU ANTIBODY AND USE THEREOF. Applicant: ADEL, INC. The sequence listing filed with the application follows.

SEQUENCE LISTING (26 sequences)

SEQ ID NO: 1 - protein, 8 aa, Artificial Sequence
  amino acid seqeunce for anti-tau antibody of CDR1 (VH)
GDSITSGY

SEQ ID NO: 2 - protein, 7 aa, Artificial Sequence
  amino acid seqeunce for anti-tau antibody of CDR2 (VH)
IRYSGRT

SEQ ID NO: 3 - protein, 7 aa, Artificial Sequence
  amino acid seqeunce for anti-tau antibody of CDR3 (VH)
ASVYFTY

SEQ ID NO: 4 - protein, 11 aa, Artificial Sequence
  amino acid seqeunce for anti-tau antibody of CDR1 (VL)
QSLLDSDGKTY

SEQ ID NO: 5 - protein, 3 aa, Artificial Sequence
  amino acid seqeunce for anti-tau antibody of CDR2 (VL)
LVS

SEQ ID NO: 6 - protein, 9 aa, Artificial Sequence
  amino acid seqeunce for anti-tau antibody of CDR3 (VL)
WQGSHFPYT

SEQ ID NO: 7 - protein, 113 aa, Artificial Sequence
  amino acid seqeunce for anti-tau antibody of variable region (VH)
EVQLEESGPSLVKPSQTLSLTCSVTGDSITSGYWNWIRKFPGNKLEYMGYIRYSGRTYYNPSLKSRISITRDTSKNQFYLQLISVTTEDTATYYCASVYFTYWGQGTLVTVSS

SEQ ID NO: 8 - protein, 113 aa, Artificial Sequence
  amino acid seqeunce for anti-tau antibody of variable region (VH)
EVQLQESGPGLVKPSQTLSLTCTVSGDSITSGYWNWIRQPPGKGLEYIGYIRYSGRTYYNPSLKSRVTISRDTSKNQFSLKLSSVTAADTAVYYCASVYFTYWGQGTLVTVSS

SEQ ID NO: 9 - protein, 113 aa, Artificial Sequence
  amino acid seqeunce for anti-tau antibody of variable region (VH)
EVQLQQSGPGLVKPSQTLSLTCAVSGDSITSGYWNWIRQSPSRGLEWLGYIRYSGRTYYNPSLKSRITINRDTSKNQFSLQLNSVTPEDTAVYYCASVYFTYWGQGTLVTVSS

SEQ ID NO: 10 - protein, 113 aa, Artificial Sequence
  amino acid seqeunce for anti-tau antibody of variable region (VH)
EVTLKESGPTLVKPTQTLTLTCTVSGDSITSGYWNWIRQPPGKALEYLAYIRYSGRTYYNPSLKSRLTITRDTSKNQVVLTMTNMDPVDTATYYCASVYFTYWGQGTLVTVSS

SEQ ID NO: 11 - protein, 113 aa, Artificial Sequence
  amino acid seqeunce for anti-tau antibody of variable region (VH)
EVQLVESGGGLVQPGRSLRLSCTVSGDSITSGYWNWFRQAPGKGLEYVGYIRYSGRTYYNPSLKSRFTISRDTSKNIAYLQMNSLKTEDTAVYYCASVYFTYWGQGTLVTVSS

SEQ ID NO: 12 - protein, 112 aa, Artificial Sequence
  amino acid seqeunce for anti-tau antibody of variable region (VL)
DVLMTQTPLTLSVTIGQPASISCKSSQSLLDSDGKTYLNWLLQRPGQSPKRLISLVSKLDSGVPDRFTGSGSGTDFTLKISRVEAEDLGVYYCWQGSHFPYTFGGGTKLEIK

SEQ ID NO: 13 - protein, 112 aa, Artificial Sequence
  amino acid seqeunce for anti-tau antibody of variable region (VL)
DVVMTQSPLSLPVTLGQPASISCKSSQSLLDSDGKTYLNWFQQRPGQSPKRLISLVSKLDSGVPDRFSGSGSGTDFTLKISRVEAEDVGVYYCWQGSHFPYTFGQGTKLEIK

SEQ ID NO: 14 - protein, 112 aa, Artificial Sequence
  amino acid seqeunce for anti-tau antibody of variable region (VL)
DVVMTQSPDSLAVSLGERATINCKSSQSLLDSDGKTYLNWYQQKPGQSPKRLISLVSKLDSGVPDRFSGSGSGTDFTLTISSLQAEDVAVYYCWQGSHFPYTFGQGTKLEIK

SEQ ID NO: 15 - protein, 112 aa, Artificial Sequence
  amino acid seqeunce for anti-tau antibody of variable region (VL)
EVVLTQSPGTLSLSPGERATLSCKSSQSLLDSDGKTYLNWYQQKPGQSPKRLISLVSKLDSGIPDRFSGSGSGTDFTLTISRLEPEDFAVYYCWQGSHFPYTFGQGTKLEIK

SEQ ID NO: 16 - DNA, 339 bp, Artificial Sequence
  nucleotide sequence of anti-tau antibody of variable region (VH)
gaggtgcagctggaggagtcaggacctagcctcgtgaaaccttctcagactctgtccctcacctgttctgtcactggcgactccatcaccagtggttactggaactggatccggaaattcccagggaataaacttgagtacatggggtacataaggtacagtggtagaacttactacaatccatctctcaaaagtcgaatctccatcactcgagacacatcaaagaaccagttctacctgcagttgatttctgtgactactgaggacacagccacatattactgtgcaagtgtttactttacttactggggccaagggactctggtcactgtctctaca

SEQ ID NO: 17 - DNA, 339 bp, Artificial Sequence
  nucleotide sequence of anti-tau antibody of variable region (VH)
gaggtgcagctgcaagaaagcggacccggtttagtgaagcccagccagactttatctttaacttgtaccgtgagcggcgactccatcaccagcggctactggaactggatcagacagcctcccggcaagggtttagagtacatcggctacattcgttacagcggtcgtacctactacaacccctctttaaagtctcgtgtgaccatctctcgtgacaccagcaagaaccagttctctttaaagctgagcagcgtgacagccgccgacacagccgtgtactactgcgccagcgtgtacttcacctactggggccaaggtactttagtgaccgtctcgagc

SEQ ID NO: 18 - DNA, 339 bp, Artificial Sequence
  nucleotide sequence of anti-tau antibody of variable region (VH)
gaggtgcagctgcagcagagcggacccggactggtgaagcccagccagacactgtctttaacttgtgccgtgagcggcgatagcatcaccagcggctactggaactggattcgtcagagccctagcagaggtttagagtggctgggctacatcagatacagcggtcgtacctactacaacccctctttaaagtctcgtatcaccatcaatcgtgacaccagcaagaaccagttctctttacagctgaacagcgtgaccccagaagacaccgccgtgtactactgcgccagcgtgtacttcacctactggggccaaggtactttagtgaccgtctcgagc

SEQ ID NO: 19 - DNA, 339 bp, Artificial Sequence
  nucleotide sequence of anti-tau antibody of variable region (VH)
gaggtgactttaaaggagagcggacccactttagtgaagcccacccagactttaactttaacttgtaccgtgagcggcgacagcatcaccagcggctactggaactggatcagacagccccccggcaaagctttagagtatttagcctacattcgttacagcggtcgtacatactacaacccctctttaaagtctcgtctgaccatcactcgtgacaccagcaagaaccaagttgtgctgaccatgaccaacatggaccccgtggacaccgccacctactactgcgccagcgtgtatttcacctactggggccaaggtactttagtgaccgtctcgagc

SEQ ID NO: 20 - DNA, 339 bp, Artificial Sequence
  nucleotide sequence of anti-tau antibody of variable region (VH)
gaggtgcagctggtggagagcggcggaggactggtgcaacccggtcgttctttaaggctgagctgcaccgtgagcggcgacagcatcacctccggctactggaactggtttcgtcaagctcccggtaaaggtttagagtacgtgggctacattcgttacagcggtcgtacctactacaatccctctttaaagtctcgtttcaccatctctcgtgacaccagcaagaacatcgcctatttacagatgaactctttaaagaccgaggacaccgccgtgtactactgcgccagcgtgtacttcacctactggggccaaggtactttagtgaccgtctcgagc

SEQ ID NO: 21 - DNA, 336 bp, Artificial Sequence
  nucleotide sequence of anti-tau antibody of variable region (VL)
gatgttttgatgacccaaactccactcactttgtcggttaccattggacaaccagcctccatctcttgcaagtcaagtcagagcctcttagatagtgatggaaagacatatttgaattggttgttacagaggccaggccagtctccaaagcgcctaatctctctggtgtctaagctggactctggagtccctgacaggttcactggcagtggatcagggacagatttcacactgaaaatcagccgagtggaggctgaggatttgggagtttattattgctggcaaggttcacattttccgtacacgttcggaggggggaccaagctggaaataaga

SEQ ID NO: 22 - DNA, 336 bp, Artificial Sequence
  nucleotide sequence of anti-tau antibody of variable region (VL)
gacgtggtgatgacccagagccctttatctttacccgttacactgggccagcccgcctctatcagctgcaagagcagccagtctttactggatagcgacggcaagacctatttaaactggttccagcagagacccggccagagccccaagaggctgatctctttagtgagcaagctggacagcggcgtgcccgatcgtttcagcggaagcggcagcggcacagacttcactttaaagatctctcgtgtggaggccgaggacgtgggcgtgtactactgctggcaaggtagccacttcccctacaccttcggccaaggtaccaagctcgagatcaag

SEQ ID NO: 23 - DNA, 336 bp, Artificial Sequence
  nucleotide sequence of anti-tau antibody of variable region (VL)
gacgtggtgatgacacagagccccgattctttagctgtgtctttaggcgagagagccaccatcaactgcaagtccagccagtctttactggacagcgacggcaagacctatttaaactggtaccagcagaagcccggccagagccccaagaggctcatctctttagtgagcaagctggacagcggcgtgcccgataggttcagcggaagcggcagcggcaccgacttcactttaaccatcagctctttacaagctgaggatgtggccgtgtactactgctggcaaggtagccacttcccctacaccttcggccaaggtaccaagctcgagatcaag

SEQ ID NO: 24 - DNA, 336 bp, Artificial Sequence
  nucleotide sequence of anti-tau antibody of variable region (VL)
gaggtggtgctgacccagagccccggtactttatctttaagccccggtgagagagccactttaagctgcaagagcagccagtctttactggacagcgacggcaagacctatttaaactggtaccagcagaagcccggccagagccccaagaggctgatctctttagtgagcaagctggacagcggcatccccgacagattcagcggaagcggcagcggcaccgacttcactttaaccatctctcgtctggagccagaagacttcgccgtgtactactgctggcaaggtagccacttcccctacaccttcggccaaggtaccaagctcgagatcaag

SEQ ID NO: 25 - protein, 441 aa, Homo sapiens
MAEPRQEFEVMEDHAGTYGLGDRKDQGGYTMHQDQEGDTDAGLKESPLQTPTEDGSEEPGSETSDAKSTPTAEDVTAPLVDEGAPGKQAAAQPHTEIPEGTTAEEAGIGDTPSLEDEAAGHVTQARMVSKSKDGTGSDDKKAKGADGKTKIATPRGAAPPGQKGQANATRIPAKTPPAPKTPPSSGEPPKSGDRSGYSSPGSPGTPGSRSRTPSLPTPPTREPKKVAVVRTPPKSPSSAKSRLQTAPVPMPDLKNVKSKIGSTENLKHQPGGGKVQIINKKLDLSNVQSKCGSKDNIKHVPGGGSVQIVYKPVDLSKVTSKCGSLGNIHHKPGGGQVEVKSEKLDFKDRVQSKIGSLDNITHVPGGGNKKIETHKLTFRENAKAKTDHGAEIVYKSPVVSGDTSPRHLSNVSSTGSIDMVDSPQLATLADEVSASLAKQGL

SEQ ID NO: 26 - protein, 129 aa, Artificial Sequence
  amino acid seqeunce for K18
QTAPVPMPDLKNVKSKIGSTENLKHQPGGGKVQIINKKLDLSNVQSKCGSKDNIKHVPGGGSVQIVYKPVDLSKVTSKCGSLGNIHHKPGGGQVEVKSEKLDFKDRVQSKIGSLDNITHVPGGGNKKIE